European Patent Specification EP 3 783 027 B1, published December 3, 2025. Title: METHOD AND COMPOSITIONS FOR INDUCING DIFFERENTIATION OF MYELOID DERIVED SUPPRESSOR CELL TO TREAT CANCER AND INFECTIOUS DISEASES. Applicant: OSE IMMUNOTHERAPEUTICS. Application EP 15794641.9. The sequence listing filed with the application follows.

SEQUENCE LISTING (10 sequences)

SEQ ID NO: 1 - DNA, 21 bp, Artificial Sequence
  Primer
ccttggtcaagcagtacagcc

SEQ ID NO: 2 - DNA, 22 bp, Artificial Sequence
  Primer
ttcgctgatgacacaaacatga

SEQ ID NO: 3 - DNA, 22 bp, Artificial Sequence
  Primer
caacaggctggataggaaacct

SEQ ID NO: 4 - DNA, 22 bp, Artificial Sequence
  Primer
tgactacgccagagttatacgc

SEQ ID NO: 5 - DNA, 20 bp, Artificial Sequence
  Primer
acagcaaaagacacccacgg

SEQ ID NO: 6 - DNA, 23 bp, Artificial Sequence
  Primer
cttgtttcattctgagcctcctc

SEQ ID NO: 7 - DNA, 22 bp, Artificial Sequence
  Primer
tcatcagggacatcatcaaacc

SEQ ID NO: 8 - DNA, 19 bp, Artificial Sequence
  Primer
cgaggaacgcacctttctg

SEQ ID NO: 9 - DNA, 22 bp, Artificial Sequence
  Primer
ggcattgctgtcctgtgattac

SEQ ID NO: 10 - DNA, 24 bp, Artificial Sequence
  Primer
ggagtagttgttagcgatgtcgta